European Patent Application EP 4 714 467 A1, published March 25, 2026. Title: がんを治療又は予防するための医薬組成物. Applicant: ISM株式会社. Application WO. The sequence listing filed with the application follows.

SEQUENCE LISTING (51 sequences)

SEQ ID NO: 1 - protein, 8 aa, unidentified
EFTFSRNG

SEQ ID NO: 2 - protein, 8 aa, unidentified
ISSGGVST

SEQ ID NO: 3 - protein, 12 aa, unidentified
CARHEGSRFAYW

SEQ ID NO: 4 - protein, 6 aa, unidentified
QDINSY

SEQ ID NO: 5 - skipped

SEQ ID NO: 6 - protein, 11 aa, unidentified
CLQYDEFPLTF

SEQ ID NO: 7 - protein, 8 aa, unidentified
GFTFNNSA

SEQ ID NO: 8 - protein, 7 aa, unidentified
ISNGGVT

SEQ ID NO: 9 - protein, 13 aa, unidentified
CARGHYPYFFDYW

SEQ ID NO: 10 - protein, 6 aa, unidentified
QDINNY

SEQ ID NO: 11 - skipped

SEQ ID NO: 12 - protein, 11 aa, unidentified
CLQYDEFPLTF

SEQ ID NO: 13 - protein, 8 aa, unidentified
GYTFTNYG

SEQ ID NO: 14 - protein, 8 aa, unidentified
INTYSGVA

SEQ ID NO: 15 - protein, 10 aa, unidentified
CARADLFAYW

SEQ ID NO: 16 - protein, 11 aa, unidentified
QSLVHSNGNTY

SEQ ID NO: 17 - skipped

SEQ ID NO: 18 - protein, 11 aa, unidentified
CSQSTHVPRTF

SEQ ID NO: 19 - protein, 145 aa, unidentified
MSTEHGPLTMNFGLSLIFLVLILKGVQCEVQLVESGGGLVKPGGSLKLSCAASEFTFSRNGMSWVRQTPAKRLEWVATISSGGVSTYYPDTVKGRFTISRDNAKNTLYLQMSSLRSEDTAMYYCARHEGSRFAYWGQGTLVTVSA

SEQ ID NO: 20 - protein, 143 aa, unidentified
MQLESSSGVLPGLSMDMRTPAQFLGILLLWFPGIKCDIKMTQSPSSMYTSLGERVTITCKASQDINSYLSWFQQKPGNSPKTLIYLVNRLVDGVPSRFSGSGSGQDYSLTIGSLEFEDVGIYYCLQYDEFPLTFGAGTKLELK

SEQ ID NO: 21 - protein, 145 aa, unidentified
MSTEHRHLTMNFGFSLIFLVLVLKGVQCEVKLVESGGGLVKPGGSLKLSCVASGFTFNNSAMSWVRQTPEKRLEWVSSISNGGVTFYPDNVKGRFTISRDDARDILYLQMSSLKSEDTAMYYCARGHYPYFFDYWGQGTTLTVSS

SEQ ID NO: 22 - protein, 129 aa, unidentified
MDMRTPAQFLGILLLWFPGIKCDIKMTQSPSSMYASLGERVTITCKASQDINNYLSWFQQKPGKSPKTLIYRANRLVDGVPSRFSGSGSGRDYSLTISSLEYEDIGIYYCLQYDEFPLTFGAGTKLELK

SEQ ID NO: 23 - protein, 134 aa, unidentified
MDWVWNLLFLMAAAQSIQAQIQLVQSGPELKKPGETVKISCKASGYTFTNYGMNWVKQAPGKGLKWMAWINTYSGVATHADDFKGRFDFSLETSASTAYLQINNLKNEDTATYFCARADLFAYWGQGTLVTVSA

SEQ ID NO: 24 - protein, 131 aa, unidentified
MKLPVRLLVLMFWIPASSSDVVMTQTPLSLPVSLGDQASISCRSSQSLVHSNGNTYLHWYLQKPGQSPKLLIYKVSNRFSGVPDRFSGSGSGTDFTLKISRVEAEDLGVYFCSQSTHVPRTFGGGTKLEIK

SEQ ID NO: 25 - protein, 117 aa, unidentified
EVQLVESGGGLVKPGGSLKLSCAASEFTFSRNGMSWVRQTPAKRLEWVATISSGGVSTYYPDTVKGRFTISRDNAKNTLYLQMSSLRSEDTAMYYCARHEGSRFAYWGQGTLVTVSA

SEQ ID NO: 26 - protein, 107 aa, unidentified
DIKMTQSPSSMYTSLGERVTITCKASQDINSYLSWFQQKPGNSPKTLIYLVNRLVDGVPSRFSGSGSGQDYSLTIGSLEFEDVGIYYCLQYDEFPLTFGAGTKLELK

SEQ ID NO: 27 - protein, 117 aa, unidentified
EVKLVESGGGLVKPGGSLKLSCVASGFTFNNSAMSWVRQTPEKRLEWVSSISNGGVTFYPDNVKGRFTISRDDARDILYLQMSSLKSEDTAMYYCARGHYPYFFDYWGQGTTLTVSS

SEQ ID NO: 28 - protein, 107 aa, unidentified
DIKMTQSPSSMYASLGERVTITCKASQDINNYLSWFQQKPGKSPKTLIYRANRLVDGVPSRFSGSGSGRDYSLTISSLEYEDIGIYYCLQYDEFPLTFGAGTKLELK

SEQ ID NO: 29 - protein, 115 aa, unidentified
QIQLVQSGPELKKPGETVKISCKASGYTFTNYGMNWVKQAPGKGLKWMAWINTYSGVATHADDFKGRFDFSLETSASTAYLQINNLKNEDTATYFCARADLFAYWGQGTLVTVSA

SEQ ID NO: 30 - protein, 112 aa, unidentified
DVVMTQTPLSLPVSLGDQASISCRSSQSLVHSNGNTYLHWYLQKPGQSPKLLIYKVSNRFSGVPDRFSGSGSGTDFTLKISRVEAEDLGVYFCSQSTHVPRTFGGGTKLEIK

SEQ ID NO: 31 - protein, 906 aa, Homo sapiens
MPLRLDIKRKLTARSDRVKSVDLHPTEPWMLASLYNGSVCVWNHETQTLVKTFEVCDLPVRAAKFVARKNWVVTGADDMQIRVFNYNTLERVHMFEAHSDYIRCIAVHPTQPFILTSSDDMLIKLWDWDKKWSCSQVFEGHTHYVMQIVINPKDNNQFASASLDRTIKVWQLGSSSPNFTLEGHEKGVNCIDYYSGGDKPYLISGADDRLVKIWDYQNKTCVQTLEGHAQNVSCASFHPELPIIITGSEDGTVRIWHSSTYRLESTLNYGMERVWCVASLRGSNNVALGYDEGSIIVKLGREEPAMSMDANGKIIWAKHSEVQQANLKAMGDAEIKDGERLPLAVKDMGSCEIYPQTIQHNPNGRFVVVCGDGEYIIYTAMALRNKSFGSAQEFAWAHDSSEYAIRESNSIVKIFKNFKEKKSFKPDFGAESIYGGFLLGVRSVNGLAFYDWDNTELIRRIEIQPKHIFWSDSGELVCIATEESFFILKYLSEKVLAAQETHEGVTEDGIEDAFEVLGEIQEIVKTGLWVGDCFIYTSSVNRLNYYVGGEIVTIAHLDRTMYLLGYIPKDNRLYLGDKELNIISYSLLVSVLEYQTAVMRRDFSMADKVLPTIPKEQRTRVAHFLEKQGFKQQALTVSTDPEHRFELALQLGELKIAYQLAVEAESEQKWKQLAELAISKCQFGLAQECLHHAQDYGGLLLLATASGNANMVNKLAEGAERDGKNNVAFMSYFLQGKVDACLELLIRTGRLPEAAFLARTYLPSQVSRVVKLWRENLSKVNQKAAESLADPTEYENLFPGLKEAFVVEEWVKETHADLWPAKQYPLVTPNEERNVMEEGKDFQPSRSTAQQELDGKPASPTPVIVASHTANKEEKSLLELEVDLDNLELEDIDTTDINLDEDILDD

SEQ ID NO: 32 - protein, 8 aa, Homo sapiens
GYTFTSYY

SEQ ID NO: 33 - protein, 8 aa, Homo sapiens
INPSTGST

SEQ ID NO: 34 - protein, 20 aa, Homo sapiens
TRGGITMVRGVSPHYYGMDV

SEQ ID NO: 35 - protein, 12 aa, Homo sapiens
QSVLYTSNNKNY

SEQ ID NO: 36 - skipped

SEQ ID NO: 37 - protein, 8 aa, Homo sapiens
QQYYRTPT

SEQ ID NO: 38 - protein, 8 aa, Homo sapiens
GFTFSSYS

SEQ ID NO: 39 - protein, 8 aa, Homo sapiens
ISSSGSYI

SEQ ID NO: 40 - protein, 18 aa, Homo sapiens
ARDHGSYYGSGSYCWFDP

SEQ ID NO: 41 - protein, 6 aa, Homo sapiens
QGISIW

SEQ ID NO: 42 - skipped

SEQ ID NO: 43 - protein, 9 aa, Homo sapiens
QQADSFPLT

SEQ ID NO: 44 - protein, 273 aa, Homo sapiens
MDWTWRVFCLLAVAPGAHSQVQLVQSGAEVKKPGASVKVSCKASGYTFTSYYLHWVRQAPGQGLEWMGIINPSTGSTMYAQKLQGSVTMTRDTSTSTVYMELSSLRSEDTAVYYCTRGGITMVRGVSPHYYGMDVWGQGTTVTVSSASTKGPSVFPLAPSSKSTSGGTAALGCLVKDYFPEPVTVSWNSGALTSGVHTFPAVLQSSGLYSLSSVVTVPSSSLGTQTYICNVNHKPSNTKVDKKVEPKSCDKTHTCPPCPAPELLGGPSVFLFP

SEQ ID NO: 45 - protein, 196 aa, Homo sapiens
MVLQTQVFISLLLWISGAYGDIVMTQSPDSLAVSQGERATINCKSSQSVLYTSNNKNYLGWYQQKPGQPPKLLIYWASTRESGVPDRFSGSGSGTDFTLTISSLQAEDVAVYYCQQYYRTPTFGGGTKVEIKRTVAAPSVFIFPPSDEQLKSGTASVVCLLNNFYPREAKVQWKVDNALQSGNSQESVTEQDSKDS

SEQ ID NO: 46 - protein, 271 aa, Homo sapiens
MELGLRWVFLVAILEGVQCEVQLVESGGGLVKPGGSLRLSCAASGFTFSSYSMHWVRQAPGKGLEWVSSISSSGSYIFYADSVRGRFTISRDNAKNSLFLQMNSLRAEDTAVYYCARDHGSYYGSGSYCWFDPWGQGTLVTVSSASTKGPSVFPLAPSSKSTSGGTAALGCLVKDYFPEPVTVSWNSGALTSGVHTFPAVLQSSGLYSLSSVVTVPSSSLGTQTYICNVNHKPSNTKVDKKVEPKSCDKTHTCPPCPAPELLGGPSVFLFP

SEQ ID NO: 47 - protein, 193 aa, Homo sapiens
MDMRVPAQLLGLLLLWFPGSRCDIQMTQSPSSVSASVGDRVTITCRASQGISIWLAWYQQKPGKAPKLLIYAASSLQSGVPSRFSGSGSGTDFTLTISSLQPEDFATYYCQQADSFPLTFGGGTKVEIKRTVAAPSVFIFPPSDEQLKSGTASVVCLLNNFYPREAKVQWKVDNALQSGNSQESVTEQDSKDS

SEQ ID NO: 48 - protein, 127 aa, Homo sapiens
QVQLVQSGAEVKKPGASVKVSCKASGYTFTSYYLHWVRQAPGQGLEWMGIINPSTGSTMYAQKLQGSVTMTRDTSTSTVYMELSSLRSEDTAVYYCTRGGITMVRGVSPHYYGMDVWGQGTTVTVSS

SEQ ID NO: 49 - protein, 112 aa, Homo sapiens
DIVMTQSPDSLAVSQGERATINCKSSQSVLYTSNNKNYLGWYQQKPGQPPKLLIYWASTRESGVPDRFSGSGSGTDFTLTISSLQAEDVAVYYCQQYYRTPTFGGGTKVEIK

SEQ ID NO: 50 - protein, 125 aa, Homo sapiens
EVQLVESGGGLVKPGGSLRLSCAASGFTFSSYSMHWVRQAPGKGLEWVSSISSSGSYIFYADSVRGRFTISRDNAKNSLFLQMNSLRAEDTAVYYCARDHGSYYGSGSYCWFDPWGQGTLVTVSS

SEQ ID NO: 51 - protein, 107 aa, Homo sapiens
DIQMTQSPSSVSASVGDRVTITCRASQGISIWLAWYQQKPGKAPKLLIYAASSLQSGVPSRFSGSGSGTDFTLTISSLQPEDFATYYCQQADSFPLTFGGGTKVEIK